European Patent Application EP 4 450 619 A1, published October 23, 2024. Title: 熱安定性に優れた逆転写酵素. Applicant: 東洋紡株式会社. The sequence listing filed with the application follows.

SEQUENCE LISTING (22 sequences)

SEQ ID NO: 1 - protein, 672 aa, Moloney murine leukemia virus
MTLNIEDEHRLHETSKEPDVSLGSTWLSDFPQAWAETGGMGLAVRQAPLIIPLKATSTPVSIKQYPMSQEARLGIKPHIQRLLDQGILVPCQSPWNTPLLPVKKPGTNDYRPVQDLREVNKRVEDIHPTVPNPYNLLSGLPPSHQWYTVLDLKDAFFCLRLHPTSQPLFAFEWRDPEMGISGQLTWTRLPQGFKNSPTLFDEALHRDLADFRIQHPDLILLQYVDDLLLAATSELDCQQGTRALLQTLGNLGYRASAKKAQICQKQVKYLGYLLKEGQRWLTEARKETVMGQPTPKTPRQLREFLGTAGFCRLWIPGFAEMAAPLYPLTKTGTLFNWGPDQQKAYQEIKQALLTAPALGLPDLTKPFELFVDEKQGYAKGVLTQKLGPWRRPVAYLSKKLDPVAAGWPPCLRMVAAIAVLTKDAGKLTMGQPLVILAPHAVEALVKQPPDRWLSNARMTHYQALLLDTDRVQFGPVVALNPATLLPLPEEGLQHNCLDILAEAHGTRPDLTDQPLPDADHTWYTDGSSLLQEGQRKAGAAVTTETEVIWAKALPAGTSAQRAELIALTQALKMAEGKKLNVYTDSRYAFATAHIHGEIYRRRGLLTSEGKEIKNKDEILALLKALFLPKRLSIIHCPGHQKGHSAEARGNRMADQAARKAAITETPDTSTLL

SEQ ID NO: 2 - protein, 672 aa, synthetic construct
  REGION 1..672: note = Reverse Transcriptase Mutant
MTLSLEDEHRLFEPSKEPDVSLGSTWIIDYPDAWAETAGLGLAVKQPPIVVELKASASPINVKQYPLSKEARDGIRPHIQKYLALGVLRPCQSAWNTPLLPVKKPGTGDYRPVQDLREVNNRVQDIHPTVPNPYNLLSTLNPERKWYTVLDLKDAFFCLPLHKDSQLLFAFEWVDPETGTSGQLTWTRLPQGFKNSPTLFDEALHRDLNNFRTQHPEVTLLQYVDDLLLAADTKENCESGTQALLSELAQLGYRASAKKAQICQQEVIFLGYSLRGGKRWLTEPRKQTVVQIPPPSNKRQLREFLGTAGFCRLWIPGFASLAAPLYPLLKGNAQFQWTPEHQQAFDNIKKALLSAPALALPDVEKPFTLYIEEKKGIARGVLTQTLGPWKRPVAYLSKKLDPVASGWPHCLKAIAAAALLIKDADKLTLGQKLTIIAPHALESIIRQPPDRWLSNSRITHYQSLLLDKDRITLGPPAPLNPATLLPESEPPVQHDCQHILAEETSIRPDLKDQPLPHPEVIWFTDGSSFLQDGKRRAGAAVVSGTKVIWSSSLPEGTSAQKAELIALTKALELAEGKRATIYTDSRYAFATAHVHGAIYQQRGLLTSAGKEIKNKDEILRLLSAVQLPKELAIVHCPGHQKGNDPVAVGNRRADEEAKLAALTETPDTSTLL

SEQ ID NO: 3 - protein, 672 aa, synthetic construct
  REGION 1..672: note = Reverse Transcriptase Mutant
MTLRLEDEYRLHQEAPPPPEDNIDRWLQEFPEAWAETGGMGLAAHRPPVLVELKPGADPVRVKQYPMSQEARKGITPHIRRLLSLGVLRPCQSAWNTPLLPVKKPHSNDYRPVQDLREVNKRVMDIHPTVPNPYTLLSSLAPSRVWYTVLDLKDAFFSLPLAPKSQPLFAFEWHDPEEGINGQLTWTRLPQGFKNSPTIFDEALHEDLGEYRREHPGLTLLQYVDDLLIAADTAEDCLQGTKDLLATLGALGYRASAKKAQICREEVSYLGYILKGGQRWLSDARKETVLKIPTPTSPREVREFLGSAGFCRLWIPGFAEIARPLYEATKEGQTFKWTEKEETAFNQIKKALLSAPALGLPDITKPFHLFVDEHKGIAKGVLTQALGPWNRPVAYLSKKLDPVAAGWPPCLRIIAATALLVKDADKLTLGQELWVTTPHAIEGVLKQPPDRWMSNARMTHYQSLLLNPPRVRFHPPAALNPATLLPDPLDAPLHDCAGILAQVHGFREDLTDRPLPDAEATWFTDGSSFVQDGQRYAGAAVVTETETVWAEALPPGTSAQRAELIALTKALTLGAGKRLNIYTDSRYAFATAHIHGAIYQERGLLTAEGKTIKNKQEILDLLAALWLPKKLAIIHCPGHQKADTPVARGNNLADQTAKAVALTSVPTTTIQL

SEQ ID NO: 4 - protein, 672 aa, synthetic construct
  REGION 1..672: note = Reverse Transcriptase Mutant
MTLSIEDEHRLHEPSKEPDVSLGSTWLSDFPQAWAETGGMGLAKQQPPLIIPLKATSTPVSVRQYPMSQEARLGIKPHIQRLLDQGILVPCQSPWNTPLLPVKKPGTNDYRPVQDLREVNKRVEDIHPTVPNPYNLLSGLPPERQWYTVLDLKDAFFCLRLHPQSQPLFAFEWRDPEMGISGQLTWTRLPQGFKNSPTLFDEALHRDLADFRIQNPQVILLQYVDDLLLAAATELDCQQGTRALLQTLGNLGYRASAKKAQICQTQVKYLGYLLRDGQRWLTEARKETVMQIPTPTTPRQLREFLGTAGFCRLWIPGFAEMAAPLYPLTKTGTLFTWGPDQQKAYQEIKQALLSAPALGLPDLTKPFELFVDEKQGYAKGVLTQKLGPWKRPVAYLSKKLDPVAAGWPPCLRMVAAIAVLTKDAGKLTLGQPLVILAPHAVEALVRQPPDRWLSNARMTHYQALLLNTDRVQFGPPVILNPATLLPEPEEPPIHDCLDILAEAHGTRPDLTDQPLPDADHTWYTDGSSLLVEGKRKAGAAVVDGKEVIWAKALPEGTSAQRAELIALTQALKMAEGKKINVYTDSRYAFATAHIHGEIYRRRGLLTSEGKEIKNKDEILALLKALHLPKRLSIIHCPGHQKGHSAEARGNRMADQAARKAALTETPDTSTLL

SEQ ID NO: 5 - DNA, 2016 bp, synthetic construct
  misc_feature 1..2016: note = G2 sequence
  source 1..2016: mol_type = other DNA
atgacgctgagccttgaagatgaacacaggctgttcgaaccgagcaaagaacccgatgtcagtctgggtagcacctggattattgactacccagatgcgtgggcagaaactgctggcttaggcttagccgtcaaacaacccccgattgtggtggaactgaaagcgtcggcaagcccgattaacgtgaagcagtatccgttatccaaagaggcacgcgatggtattcggccacacattcagaagtatctcgcgttaggtgttttgcgcccatgtcagtcggcatggaacacgccgttgctgccggtgaaaaagccgggtaccggtgattacagacccgttcaagatctgcgcgaagtgaataaccgcgttcaggatatccatccaacagtgccaaatccgtacaatctgctgtctactctaaatccggagcgcaaatggtacaccgtgttagacctgaaagacgcgttcttttgcctgccgctgcacaaagactcacagctgctgttcgcgtttgaatgggttgaccccgaaacaggtacgtcagggcagcttacttggacccgtttacctcagggattcaaaaactctccgaccctgtttgacgaagctctgcatcgagatctgaacaatttccgtacccaacatccagaagtaaccctcctgcagtacgtcgatgatctcttattggcggccgataccaaagagaactgcgaatctgggacccaagcccttctgagtgaattggcgcaactcggctatcgagcttctgcgaagaaagcgcagatatgccaacaggaagtaatcttcctcgggtattccttacgcggtggcaaacgctggttaacagaaccccgtaaacagaccgtcgtccagattccgccaccttcgaacaaacgccagctgcgtgagtttctgggtactgccggtttctgtcgcctgtggattccgggatttgcgagcttggcggctccgctgtatccactgttgaaaggcaatgcgcagtttcagtggacgcctgaacaccaacaagcgttcgataacatcaaaaaagccctcctgtcagccccggctttggccctgccggatgtcgaaaagccgtttaccctgtatattgaggagaaaaaagggatcgcccgcggagtgctgacgcagactctggggccttggaaacgtccagttgcttacctgtccaagaagctggaccccgtagcaagcggctggccgcattgtctgaaagccattgcggcagcagcgctgttgatcaaagatgcagacaagctgacgcttggccagaaactgacgatcattgctccgcatgcactggagagcattatccgtcaacctccggatcgctggctgtctaattcgcggatcacccactatcaatccttgctgcttgataaagaccggatcacactgggccctccagccccgctgaatcctgctacgctcttgcccgaaagtgaaccgccggtacagcatgattgccagcacatcctcgcggaagaaacctcgatacgtccggatctgaaagaccagccactccctcatcctgaggttatttggtttacggatggctcctcgtttcttcaggatggaaaacgtcgtgcgggtgccgcagttgttagcggcacaaaggtaatttggagctcctcactgccggaaggcaccagtgcgcagaaagcggagcttatcgcgttaaccaaagccctagaactagccgaagggaaacgcgcaaccatctatacggattcacgctatgcgtttgcgactgcccatgtgcatggtgccatctaccagcaacgtggccttttaaccagtgcaggcaaagagatcaagaacaaagacgagattctgcgtctgctgagtgctgtgcaattgccgaaagaactcgccattgtgcattgtccgggccaccagaaaggtaacgacccggtcgcagtgggcaatcgtcgtgcagacgaagaggcgaaattggctgcccttaccgaaactccggatacgagcacactgtta

SEQ ID NO: 6 - DNA, 2016 bp, synthetic construct
  misc_feature 1..2016: note = G6 sequence
  source 1..2016: mol_type = other DNA
atgaccctgcggttggaggatgagtatcgactgcatcaggaggctccgcctcctcccgaagacaacattgatcgctggctgcaggagtttccggaagcttgggcggaaaccggcggtatgggtctggccgcacatcgtccgccggtactggttgaattgaagccgggtgccgatcctgtgcgtgtcaagcaatatccgatgtctcaggaagcgcgcaaagggattaccccgcatattcgacgtctgctgtccttaggcgtacttcgcccatgccagagtgcatggaatactccgcttctccccgtcaaaaaaccgcactcgaatgactatcgtccggtccaagatctgcgcgaagtgaataaacgcgtgatggacattcacccgactgtccccaatccgtataccctcctcagctcgctggccccgagtcgtgtctggtacacggttctggacctgaaagatgcgttcttttccctgccgttagcaccgaaaagccaaccgctgtttgctttcgaatggcacgatcctgaggaagggatcaacggtcagttaacctggacacgcctgccccaaggctttaagaacagtccgaccatcttcgatgaggccctacatgaagatctgggcgaataccgccgtgaacatccaggccttactctcctgcaatacgtggatgatctgcttatcgcggccgatactgcggaagactgccttcagggtaccaaagatctgcttgcaacgctaggtgccttgggctatcgcgcatcagcgaagaaagcgcagatttgccgggaggaagtgtcgtatctgggctatattctgaaggggggacagcgttggctgagcgatgcacgtaaagaaaccgtgctgaaaattccgactccgacaagcccgagagaagtgcgcgaattcctcggttctgcagggttttgtcggctgtggattcccggttttgccgaaatcgcgaggccattatacgaagcgaccaaagaaggccagacgtttaaatggaccgagaaagaagagacggcgttcaatcagatcaaaaaagcgctgctgtctgctccggcgttaggtttgccggacattacgaaaccgtttcaccttttcgtggatgagcacaaaggtatcgcgaaaggcgtccttacccaggcgctgggaccatggaaccgtcccgtagcttacctgagcaaaaaactggacccggttgccgcgggatggccaccgtgcttacgcatcattgcagcaaccgccttgttagttaaagacgcggacaagctgaccctcggccaggagctctgggtaaccacgccacatgcgattgagggagttctgaaacagccaccagatcgctggatgtcgaacgctcgcatgacgcattaccagtcactgctcctgaatcccccacgggttcgcttccatccaccggcggcgttgaaccctgccacgctgttacctgatccgctggatgcgccgttacatgattgtgctggcatcttggcacaagtgcatggtttccgtgaagaccttaccgatcgtcctttaccggatgccgaagccacgtggtttaccgatggcagcagctttgtgcaagatggtcaacgctatgctggcgcagcagtcgtgaccgaaacggaaacagtatgggccgaagctttgcctccggggacttcagcgcaacgtgcggaactgatcgcgctgaccaaagccttgacactgggtgcaggcaaacgtctgaacatttacacagactcccgttatgcctttgcaacagcccacatacatggtgccatctatcaggaacgcggcctattgacggcggaaggcaagactatcaaaaacaagcaagagatactggacttactcgctgcgctgtggctgcctaagaaactggccatcattcactgtcctggccaccagaaagccgataccccggttgctcgtgggaacaatttagccgaccagacggctaaagcggtggcactgaccagtgttccaactacgaccattcagttg

SEQ ID NO: 7 - DNA, 24 bp, synthetic construct
  misc_feature 1..24: note = primer
  source 1..24: mol_type = other DNA
gttcgaccgtcttctcagcgctcc

SEQ ID NO: 8 - DNA, 25 bp, synthetic construct
  misc_feature 1..25: note = primer
  source 1..25: mol_type = other DNA
gccatgcatgtctgagtacgcacgg

SEQ ID NO: 9 - DNA, 25 bp, synthetic construct
  misc_feature 1..25: note = primer
  source 1..25: mol_type = other DNA
tctagaattaccacagttatccaag

SEQ ID NO: 10 - DNA, 2016 bp, synthetic construct
  misc_feature 1..2016: note = G7 sequence
  source 1..2016: mol_type = other DNA
atgacgctctcaatcgaagatgagcaccggttgcatgaaccgagcaaagaacccgacgtgtctctgggctctacgtggttaagcgactttccacaagcctgggctgaaaccggtggcatgggcctcgccaaacaacagcctccgctgatcataccgctgaaggctacctccacacccgtttcagtgcgtcaatatccgatgagtcaggaagcccggctgggtattaaaccgcacattcagcggttgttggaccaaggcattctggtaccgtgtcaatcaccgtggaatactccccttttaccggtcaaaaaaccgggtaccaacgactatcgcccagttcaggacttgcgcgaggtgaacaaacgtgtagaggacattcacccgaccgttccaaacccgtacaacttgctgtccggtttgcctccagaacgacagtggtatacggtgctggatctgaaagatgcattcttttgcctgcgtttacacccccagagccaaccgctgtttgcgttcgaatggcgtgacccggaaatgggcattagcggacagcttacctggactcgactacctcagggcttcaagaactcgccgacgctgttcgatgaagcactgcatcgcgatctggccgattttcgcattcaaaacccacaggtaatccttctgcaatacgtggatgatctgctgttagcggcagctaccgagctcgattgccaacagggcactcgtgcgctgttacagacactgggcaatctgggctatcgtgcatccgccaaaaaggcgcagatttgccaaacccaagtgaaatacctcggctatttactgcgtgatggtcagcgttggctgaccgaagcccgtaaagaaaccgtcatgcagattccgaccccgacgactccacgccagctccgcgaattccttggcaccgcgggtttctgtcgtctgtggattccggggtttgcagagatggcagcgccgctgtaccccttgacgaaaaccgggactctgtttacctgggggccggatcagcagaaagcgtatcaggagatcaaacaggcgcttctgagtgccccggcattgggtttgcccgatctcacgaaaccgttcgagctatttgtagatgagaaacaggggtatgcgaaaggcgtccttacgcagaaactgggtccgtggaaacgcccggttgcttatctgtcgaagaaacttgatcctgttgcggcgggatggccgccgtgtctgcgcatggtggctgccatagcggtgctgaccaaagacgccggtaaactgactctgggacagccattagtcatcctggcccctcatgccgtcgaagcgctggttcgccaacctccagatcgttggctctcgaatgcgcgtatgacgcactatcaggcgctgctgctgaataccgaccgtgtgcagtttggtcctccggttatcctgaatccagcaacgctcctcccggagccggaagaacctcctattcacgactgccttgacattctggcggaagctcatggtacacgcccagatctgaccgatcagccgttaccggacgcggatcatacgtggtacacggatgggagctctttactagtagaaggcaaacgcaaagctggagcagcagtggtcgacggcaaagaagtgatttgggctaaagcgttaccagaaggcaccagtgcccagagagcagagttgattgccttgacccaagcgctgaaaatggccgaaggcaagaagattaacgtttacacagatagccggtatgcatttgcgaccgctcacatccatggtgagatctaccgtcgcaggggtttactgactagtgaagggaaagaaatcaagaacaaggatgaaatcctggcgctgcttaaagccctgcatctccctaaacgcctgtccatcatccattgtcccggtcatcagaagggccatagcgctgaagcccgtggaaatcgcatggcggatcaagcagcacgcaaagccgcgctgactgaaacaccggatacatcgaccttattg

SEQ ID NO: 11 - DNA, 23 bp, synthetic construct
  source 1..23: mol_type = other DNA
aactcacgctatgcgtttgcgac

SEQ ID NO: 12 - DNA, 23 bp, synthetic construct
  source 1..23: mol_type = other DNA
cgtatagatggttgcgcgtttcc

SEQ ID NO: 13 - DNA, 30 bp, synthetic construct
  source 1..30: mol_type = other DNA
aactgtgtaaatgttcagacgtttgcctgc

SEQ ID NO: 14 - DNA, 27 bp, synthetic construct
  source 1..27: mol_type = other DNA
tgtgtaaatgttcagacgtttgcctgc

SEQ ID NO: 15 - DNA, 20 bp, synthetic construct
  source 1..20: mol_type = other DNA
agaaaatctggcaccacacc

SEQ ID NO: 16 - DNA, 20 bp, synthetic construct
  source 1..20: mol_type = other DNA
agaggcgtacagggatagca

SEQ ID NO: 17 - DNA, 17 bp, synthetic construct
  source 1..17: mol_type = other DNA
cctccggcccctgaatg

SEQ ID NO: 18 - DNA, 18 bp, synthetic construct
  source 1..18: mol_type = other DNA
accggatggccaatccaa

SEQ ID NO: 19 - DNA, 26 bp, synthetic construct
  source 1..26: mol_type = other DNA
ccgactactttgggtgtccgtgtttc

SEQ ID NO: 20 - DNA, 17 bp, synthetic construct
  source 1..17: mol_type = other DNA
gtgaccctgccgttgca

SEQ ID NO: 21 - DNA, 32 bp, synthetic construct
  source 1..32: mol_type = other DNA
gttatgatcagagagagaagaattagcaatag

SEQ ID NO: 22 - DNA, 27 bp, synthetic construct
  source 1..27: mol_type = other DNA
tatgccggcgatccaacctcccttata